European Patent Specification EP 3 681 271 B1, published July 31, 2024. Title: A METHOD FOR PRODUCING BANANA PLANTS WITH TOLERANCE TO FUSARIUM OXYSPORUM CUBENSIS TR4. Applicant: RAHAN MERISTEM (1998) Ltd. The sequence listing filed with the application follows.

SEQUENCE LISTING (1 sequence)

SEQ ID NO: 1 - DNA, 309 bp, Artificial Sequence
  Ban-1 probe
ggaggaggatgtatatgatgcaacctgagggattcatgtccaagaactgcccagataaggtgtgtaggttgcttagatccatttagggactaaagcaagcttcccgaagttggaacataagatttgatgaggcaatcagatcttatgacttcgttaagaacgaagatgagccttgtgtatacagaaaggtaagtgggagcgctattagctttttggtgttatatgtagatgacatcctcgtctttgggaatgacataggaatgctatccacaataaaggcttggttatctagacacttctccatgaagg